European Patent Specification EP 3 215 615 B1, published May 21, 2025. Title: POLYPEPTIDES HAVING PROTEASE ACTIVITY. Applicant: Novozymes A/S. The sequence listing filed with the application follows.

SEQUENCE LISTING (20 sequences)

SEQ ID NO: 1 - DNA, 1212 bp, Janibacter sp. HTCC2649
  CDS (1)..(1209)
  sig_peptide (1)..(90)
  mat_peptide (601)..(1209)
atgtctcgcagaagtctcaccgtcctggccggaaccctctcggccgctgcagcagcaaccgccctctgcgtcgcgcccgccgcgaacgctgcgaaccctggcccgagcggcccgagcagcccgagcaccggacccctggctgtcgactccggtgactccgtcgccgagatgtcggcgcagtggctcgcgacggaggagggcctgagcctcgagaccgcccgtgaccgagtggccgctcaggaggggttgtcgcgcacggcgacgtcgctggagacgtcgctcggcgccaaggccgtcggcacgtggatcgaccaggcgacgggcgtgctccacgtcaacgtcaccgacgccgccgccgcgtccacggtgcgttccgccggggcgagcgcccgtgtcgtcagcgccgacaagtcccggctcgccgcctccgagaaggccgccaccaccgtcgccggcaaggacaccatcgcgtcctacgtcgacccggtcaccaacaaggtcatcctcacggtgcccgcggatcgcgtcgaggcgacccgcgccaagatcgccgacccgtccgtcacggtcgagggcacgcaggccaaggtctccacccaggccaacgtctacggcggccagcagatcgagttcagcggctacgtctgctcgctcggcttcaacgccaccaaggccggcgccccggtcttcatcacggccggccactgcggcgagggctaccagaccttctccaagaacggcacgaccctgggcaagacacaggccttctcgttccccggcaacgactacgcctactcgaccctcgcgtcgagctggaccggcatcggcgcggtcgacctgtggaccggctccgcacgggcggtgacggggtcgagcaacgccgccgtcggcaccgcgatctgcaagtccggccgcaccacctactggacctgcggctcggtccaggccaagaacgtcaccgtgaactacgacaacggtgacggcacgacgagctcggtctcgggcctcacgaagtccaacacctgcaccgagggcggcgactccggcggctcctggatggcgggcaaccttgcccagggcgtgacgagcggcggcgcgggctacggctccagcggagtgtgcggcgagaaggtcggccagcccaacatcgcctacttccagccggtcggcgagatcctctccgcctacggcctcaccctcaagacggcctga

SEQ ID NO: 2 - protein, 403 aa, Janibacter sp. HTCC2649
MSRRSLTVLAGTLSAAAAATALCVAPAANAANPGPSGPSSPSTGPLAVDSGDSVAEMSAQWLATEEGLSLETARDRVAAQEGLSRTATSLETSLGAKAVGTWIDQATGVLHVNVTDAAAASTVRSAGASARVVSADKSRLAASEKAATTVAGKDTIASYVDPVTNKVILTVPADRVEATRAKIADPSVTVEGTQAKVSTQANVYGGQQIEFSGYVCSLGFNATKAGAPVFITAGHCGEGYQTFSKNGTTLGKTQAFSFPGNDYAYSTLASSWTGIGAVDLWTGSARAVTGSSNAAVGTAICKSGRTTYWTCGSVQAKNVTVNYDNGDGTTSSVSGLTKSNTCTEGGDSGGSWMAGNLAQGVTSGGAGYGSSGVCGEKVGQPNIAYFQPVGEILSAYGLTLKTA

SEQ ID NO: 3 - DNA, 1203 bp, Artificial Sequence
  Synthetic construct
  CDS (1)..(1200)
  sig_peptide (1)..(81)
  mat_peptide (592)..(1200)
atgaagaaaccgttggggaaaattgtcgcaagcaccgcactactcatttctgttgcttttagttcatcgatagcatcggctgcaaatccgggaccgagcggaccgtcatcaccgtcaacaggaccgctggcagttgattcaggcgattcagttgcagaaatgtcagcacaatggctggcaacagaagaaggcctgtcactggaaacagcaagagatagagttgcagcacaagaaggactttcaagaacagcaacatcacttgaaacaagccttggcgcaaaagcagttggcacatggattgatcaagcaacaggcgttctgcatgttaatgttacagatgcagcagcagcatcaacagttagatcagcaggcgcatcagcaagagttgtttcagcagataaatcaagactggcagcatcagaaaaagcagcgacaacagttgcaggcaaagatacaattgcatcatatgttgatccggtcacgaacaaagttattctgacagttccggcagatagagtcgaagcaacacgcgcaaaaattgcagatccgtcagttacagttgaaggcacacaagcaaaagtttcaacacaagcgaatgtttatggcggacagcaaattgaatttagcggctatgtttgctcactgggctttaatgcaacaaaagcaggcgctccggtctttattacagcaggccattgcggagaaggctatcaaacattttcaaaaaatggcacaacactgggcaaaacacaggcattttcatttccgggaaacgattatgcatattcaacacttgcatcaagctggacaggcattggcgcagttgatctgtggacaggctcagcgagagcagttacaggctcatcaaatgcagcagttggaacagcaatttgcaaaagcggcagaacaacatattggacatgcggctcagttcaagcaaaaaatgtgacagtcaactatgataatggcgacggcacaacatcatcagtttcaggccttacaaaaagcaacacatgcacagaaggcggagatagcggaggctcatggatggcaggcaatctggcacaaggcgttacatcaggcggagcaggatatggctcatcaggcgtctgcggagaaaaagttggacaaccgaatattgcatattttcaaccggtcggcgaaattctgtcagcatatggcctgacacttaaaacagcataa

SEQ ID NO: 4 - protein, 400 aa, Artificial Sequence
  Synthetic Construct
MKKPLGKIVASTALLISVAFSSSIASAANPGPSGPSSPSTGPLAVDSGDSVAEMSAQWLATEEGLSLETARDRVAAQEGLSRTATSLETSLGAKAVGTWIDQATGVLHVNVTDAAAASTVRSAGASARVVSADKSRLAASEKAATTVAGKDTIASYVDPVTNKVILTVPADRVEATRAKIADPSVTVEGTQAKVSTQANVYGGQQIEFSGYVCSLGFNATKAGAPVFITAGHCGEGYQTFSKNGTTLGKTQAFSFPGNDYAYSTLASSWTGIGAVDLWTGSARAVTGSSNAAVGTAICKSGRTTYWTCGSVQAKNVTVNYDNGDGTTSSVSGLTKSNTCTEGGDSGGSWMAGNLAQGVTSGGAGYGSSGVCGEKVGQPNIAYFQPVGEILSAYGLTLKTA

SEQ ID NO: 5 - protein, 203 aa, Janibacter sp. HTCC2649
  mat_polypeptide (1)..(203)
ANVYGGQQIEFSGYVCSLGFNATKAGAPVFITAGHCGEGYQTFSKNGTTLGKTQAFSFPGNDYAYSTLASSWTGIGAVDLWTGSARAVTGSSNAAVGTAICKSGRTTYWTCGSVQAKNVTVNYDNGDGTTSSVSGLTKSNTCTEGGDSGGSWMAGNLAQGVTSGGAGYGSSGVCGEKVGQPNIAYFQPVGEILSAYGLTLKTA

SEQ ID NO: 6 - protein, 27 aa, Artificial Sequence
  Bacillus clausii secretion signal
MKKPLGKIVASTALLISVAFSSSIASA

SEQ ID NO: 7 - DNA, 1596 bp, Nocardiopsis sp.
  CDS (318)..(1463)
  sig_peptide (318)..(404)
  mat_peptide (900)..(1463)
acgtttggtacgggtaccggtgtccgcatgtggccagaatgcccccttgcgacagggaacggattcggtcggtagcgcatcgactccgacaaccgcgaggtggccgttcgcgtcgccacgttctgcgaccgtcatgcgacccatcatcgggtgaccccaccgagctctgaatggtccaccgttctgacggtctttccctcaccaaaacgtgcacctatggttaggacgttgtttaccgaatgtctcggtgaacgacaggggccggacggtattcggccccgatcccccgttgatccccccaggagagtagggaccccatgcgaccctcccccgttgtctccgccatcggtacgggagcgctggccttcggtctggcgctgtccggtaccccgggtgccctcgcggccaccggagcgctcccccagtcacccaccccggaggccgacgcggtctccatgcaggaggcgctccagcgcgacctcgacctgacctccgccgaggccgaggagctgctggccgcccaggacaccgccttcgaggtcgacgaggccgcggccgaggccgccggggacgcctacggcggctccgtcttcgacaccgagagcctggaactgaccgtcctggtcaccgatgccgccgcggtcgaggccgtggaggccaccggcgccgggaccgagctggtctcctacggcatcgacggtctcgacgagatcgtccaggagctcaacgccgccgacgccgttcccggtgtggtcggctggtacccggacgtggcgggtgacaccgtcgtcctggaggtcctggagggttccggagccgacgtcagcggcctgctcgcggacgccggcgtggacgcctcggccgtcgaggtgaccacgagcgaccagcccgagctctacgccgacatcatcggtggtctggcctacaccatgggcggccgctgttcggtcggcttcgcggccaccaacgccgccggtcagcccgggttcgtcaccgccggtcactgcggccgcgtgggcacccaggtgaccatcggcaacggcaggggcgtcttcgagcagtccgtcttccccggcaacgacgcggccttcgtccgcggtacgtccaacttcacgctgaccaacctggtcagccgctacaacaccggcgggtacgccacggtcgccggtcacaaccaggcccccatcggctcctccgtctgccgctccggctccaccaccggttggcactgcggcaccatccaggcccgcggccagtcggtgagctaccccgagggcaccgtcaccaacatgacccggaccaccgtgtgcgccgagcccggcgactccggcggctcctacatctccggcacccaggcccagggcgtgacctccggcggctccggcaactgccgcaccggcgggaccaccttctaccaggaggtcacccccatggtgaactcctggggcgtccgtctccggacctgatccccgcggttccaggcggaccgacggtcgtgacctgagtaccaggcgtccccgccgcttccagcggcgtccgcaccggggtgggaccgggcgtggccacggccccacccgtgaccggaccgcccggcta

SEQ ID NO: 8 - protein, 382 aa, Nocardiopsis sp.
MRPSPVVSAIGTGALAFGLALSGTPGALAATGALPQSPTPEADAVSMQEALQRDLDLTSAEAEELLAAQDTAFEVDEAAAEAAGDAYGGSVFDTESLELTVLVTDAAAVEAVEATGAGTELVSYGIDGLDEIVQELNAADAVPGVVGWYPDVAGDTVVLEVLEGSGADVSGLLADAGVDASAVEVTTSDQPELYADIIGGLAYTMGGRCSVGFAATNAAGQPGFVTAGHCGRVGTQVTIGNGRGVFEQSVFPGNDAAFVRGTSNFTLTNLVSRYNTGGYATVAGHNQAPIGSSVCRSGSTTGWHCGTIQARGQSVSYPEGTVTNMTRTTVCAEPGDSGGSYISGTQAQGVTSGGSGNCRTGGTTFYQEVTPMVNSWGVRLRT

SEQ ID NO: 9 - protein, 415 aa, Austwickia chelonae NBRC 105200
MNKRIGATLALLSSAALLPAAAPLTAQAADEKKSEELSTIQEMSAEWLSKSYGLDGEEAKRRVKDQDGHAQKAKDIEGDLGDKTAGSFIDQKRGKLVVTVTDEKAVDKVKEKDKNADVRVVKNSASKLNDSKKNAEDKVGDKMAASYVDVERNVVVLTVPKDKAEEAKKQVKDVQGVEVQEVEATIEAQANLYGGQEIQFGRSVCSVGFPATKDGKNVFITAGHCAAGGQAFRRNGQNLGKPVKYNFPGPDMAYSTMENGWNGVGAVDHWNGKAVAVAGSQEAPVGATVCKSGRTTRWTCGVIQAKNVTVRYGKPGGGQDIVRGMTQANVCSEGGDSGGSWIAGNQAQGVTSGGAGYGPNKSCGEKVGRPNVAYFQPLNPILKDYGLKLTTHNGGKGGGDNGGDRNRDNRKGGRY

SEQ ID NO: 10 - DNA, 1203 bp, Terracoccus sp.
  CDS (1)..(1200)
  sig_peptide (1)..(78)
  mat_peptide (589)..(1200)
atgatccgcaccagtctcaccaccctggccgccacggccgcgatcgccaccgcgatcaccgtgatgccggcccaggcatcgaccctcgcgtccgacccgacccccgcgccgacgccagcggcgtccaccgactcaggccagtccgtcgccgagatgtcggcgcgctggctcgcgaaggaccgtgccatcagcctcgccacggctcgccagcgcgtcgcggcccaggacggacagacccgcacggcggcctcgctcgagcgcgcgctcggcgcccgggccgcagggtcctacatcgacgccacctccggcgcgctcgtcgtcaacgtcgtcgacaccgcgtccgtcgccagggtgctgtctgccggtgccgtcgccaaggtcgtcgaccgctcgacgagcgagctgtccgcgaccgagcgcgcggcacgcgcacgtgccgggtcggccgtcgtgtcctcctacaccgaccccgtcaccaacggcgtcgtcctgaccgtccccagcgcgcgggtctcggaggtccgcagcgaggtcgttggtctcgacggggtgaccgtcgcaggcaccgacgcacggacgacgacgcaggccaacgtctacggcggccagcagatcgagttcagcggctacgtctgctcgctcggcttcaacgccacccgcggcggtgctccggtgttcgtcaccgccggccactgtggtgagggttaccagaccttcagcaagggaggcacgacgctggggtcgacgcaggcgtactccttcccgggcaacgactacgcctactcgaccctgacgtcgagctggaccggggtcggtgccgtcgacctctacgacggcgtcaacgcccgccgggtctcgggctactcgaacgccccggtcgggaccgcgatctgcaagtcgggccgcacgaccggctggacctgcggctcggtgcaggccaagaacgtcaccgtcaactacagcaacgccgacggctcgacgagcaccgtgagcggcctgacgaagagcaacacctgcaccgagggtggcgactcgggcggctcgtggatggcgagcacgtcggcacagggcgtgacgagcggtggtgccggctacggcgccaacagcgtctgcggccagaaggtcggccagcccaacatcgcctacttccagcccgtcgacgagatcgtgtcggcctacggcctgacgctcaagacctcctga

SEQ ID NO: 11 - protein, 400 aa, Terracoccus sp.
MIRTSLTTLAATAAIATAITVMPAQASTLASDPTPAPTPAASTDSGQSVAEMSARWLAKDRAISLATARQRVAAQDGQTRTAASLERALGARAAGSYIDATSGALVVNVVDTASVARVLSAGAVAKVVDRSTSELSATERAARARAGSAVVSSYTDPVTNGVVLTVPSARVSEVRSEVVGLDGVTVAGTDARTTTQANVYGGQQIEFSGYVCSLGFNATRGGAPVFVTAGHCGEGYQTFSKGGTTLGSTQAYSFPGNDYAYSTLTSSWTGVGAVDLYDGVNARRVSGYSNAPVGTAICKSGRTTGWTCGSVQAKNVTVNYSNADGSTSTVSGLTKSNTCTEGGDSGGSWMASTSAQGVTSGGAGYGANSVCGQKVGQPNIAYFQPVDEIVSAYGLTLKTS

SEQ ID NO: 12 - DNA, 1206 bp, Artificial Sequence
  Expression construct
  CDS (1)..(1203)
  sig_peptide (1)..(81)
  mat_peptide (592)..(1203)
atgaagaaaccgttggggaaaattgtcgcaagcaccgcactactcatttctgttgcttttagttcatcgatcgcatcggcttcaacactggcatcagatccgacaccggcacctacaccggcagcaagcacagattcaggccaatcagttgcagaaatgtcagcaagatggctggcaaaagatagagcaatttcactggcaacagcaagacagcgcgttgcagcacaagatggccaaacaagaacagcagcatcactggaaagagcacttggcgcaagagcagcaggctcatatattgatgcaacatcaggcgcactggttgttaatgttgttgatacagcaagcgttgcaagagttctgtcagcaggcgcagttgcaaaagttgtcgatagatcaacatcagaactgagcgcaacagaaagagcggcaagagcgagagcaggcagcgcagttgtttcatcatatacagatccggttacaaatggcgttgttctgacagttccgagcgcaagagtttcagaagttagaagcgaagttgttggcctggatggcgttacagttgcaggcacagatgcaagaacaacaacacaagcaaatgtttatggcggacagcagattgaattttcaggctatgtttgctcactgggctttaatgcaacaagaggcggagcaccggtttttgttacagcaggccattgcggagaaggctatcaaacattttcaaaaggcggaacaacactgggcagcacacaagcatattcatttccgggaaacgattatgcatatagcacactgacatcatcatggacaggcgttggagcagttgatctgtatgatggcgtcaatgcaagaagagttagcggctattcaaatgcaccggttggcacagcaatttgcaaaagcggcagaacaacaggctggacatgcggctcagttcaagcaaaaaatgtcacagtcaattatagcaatgcagatggctcaacatcaacagtttcaggccttacaaaaagcaacacatgcacagaaggcggagatagcggaggctcatggatggcatcaacaagcgcacaaggcgttacaagcggaggcgcaggctatggcgcaaattcagtttgcggacaaaaagttggacaaccgaacattgcatattttcaaccggtcgatgaaattgttagcgcatatggcctgacactgaaaacatcataa

SEQ ID NO: 13 - protein, 401 aa, Artificial Sequence
  Synthetic Construct
MKKPLGKIVASTALLISVAFSSSIASASTLASDPTPAPTPAASTDSGQSVAEMSARWLAKDRAISLATARQRVAAQDGQTRTAASLERALGARAAGSYIDATSGALVVNVVDTASVARVLSAGAVAKVVDRSTSELSATERAARARAGSAVVSSYTDPVTNGVVLTVPSARVSEVRSEVVGLDGVTVAGTDARTTTQANVYGGQQIEFSGYVCSLGFNATRGGAPVFVTAGHCGEGYQTFSKGGTTLGSTQAYSFPGNDYAYSTLTSSWTGVGAVDLYDGVNARRVSGYSNAPVGTAICKSGRTTGWTCGSVQAKNVTVNYSNADGSTSTVSGLTKSNTCTEGGDSGGSWMASTSAQGVTSGGAGYGANSVCGQKVGQPNIAYFQPVDEIVSAYGLTLKTS

SEQ ID NO: 14 - protein, 204 aa, Terracoccus sp.
  mat_peptide (1)..(204)
ANVYGGQQIEFSGYVCSLGFNATRGGAPVFVTAGHCGEGYQTFSKGGTTLGSTQAYSFPGNDYAYSTLTSSWTGVGAVDLYDGVNARRVSGYSNAPVGTAICKSGRTTGWTCGSVQAKNVTVNYSNADGSTSTVSGLTKSNTCTEGGDSGGSWMASTSAQGVTSGGAGYGANSVCGQKVGQPNIAYFQPVDEIVSAYGLTLKTS

SEQ ID NO: 15 - protein, 9 aa, Artificial Sequence
  Motif VCG[E/Q]KVGQP.
  MISC_FEATURE (4)..(4): The amino acid in position 4 of the conserved motif is either glutamic acid (Glu, E) or Glutamine (Gln, Q).
VCGXKVGQP

SEQ ID NO: 16 - DNA, 1209 bp, Knoellia flava
  CDS (1)..(1206)
  sig_peptide (1)..(87)
  mat_peptide (595)..(1206)
atgtctcgcagacgtctcaccgtcctcgccgggggcctctcggccgcggcggcagccaccgccctctgcgtcgcgcccgcgtccgccgccacctccgcggcgggcggtccggagccgagcaccggccctctcgccaccgactcgggcgcgtccgtcgccgagatgtcggcccggtggctcgccaaggagcacgacctgagcatcgagaccgctcgtgagcggatcgcgtcccaggaggacaagagtcgcaaggccgaggctctcgaacggtcgctcggcgcgcgagccgtgggctcgttcatcgaccagaccggcggcgtgctcgtcgtcaacgtcaccgacgccgacgccgctgcccgcgtgcagaaggcgggcgcgaccgcccgcgtcgtcaccgaggacaaggcggagctcggcgcgtcgcaggcgagggcggtcaaggcgctcggcgccacggtcatcgacagctccgtcgacccggtgaccaacaaggtcgtcgtcaccgtgcccaccgccgacgtcgccgccgcgcgggcgcgcacgagcgacccgtcggtgacgatccagggcaccgacgcgacggtgtcgacgcaggccaacgtctatggcgggcagcagatcgagttcagcggctacgtctgctcgctgggcttcaacgcgacgaagtccggcaccccggtcttcatcaccgccggccactgcgccgaggggaaccagaccttcacgcgcaacggcacgaccctcggcacgacccgcggctggtccttcccgggcaacgactacgcctactcgagcctcacctcgagctggaccggcatcggcgccgtcgacctgtggaacggcacgagcgcgcgctccgtcacgggctcgagcaacgccgccgtcggcaccgcgatctgcaagtcgggccgcacgaccggctggacctgtggctcggtccagaccaagaacgtcaccgtcaactacaacaacggcgacggcacctactcgaccgtgagcggcctgacgaagtccaacacctgcaccgagggtggcgactccggcggctcgtggatggcgggcaacctcgcccagggcgtgacgagcggcggcgccggctacggctccaacggcgtctgcggccagaaggtcggccagcccaacatcgcctacttccagccgatcggcgagatcctctccgtctacggcctcaccctcaagaccgcctga

SEQ ID NO: 17 - protein, 402 aa, Knoellia flava
MSRRRLTVLAGGLSAAAAATALCVAPASAATSAAGGPEPSTGPLATDSGASVAEMSARWLAKEHDLSIETARERIASQEDKSRKAEALERSLGARAVGSFIDQTGGVLVVNVTDADAAARVQKAGATARVVTEDKAELGASQARAVKALGATVIDSSVDPVTNKVVVTVPTADVAAARARTSDPSVTIQGTDATVSTQANVYGGQQIEFSGYVCSLGFNATKSGTPVFITAGHCAEGNQTFTRNGTTLGTTRGWSFPGNDYAYSSLTSSWTGIGAVDLWNGTSARSVTGSSNAAVGTAICKSGRTTGWTCGSVQTKNVTVNYNNGDGTYSTVSGLTKSNTCTEGGDSGGSWMAGNLAQGVTSGGAGYGSNGVCGQKVGQPNIAYFQPIGEILSVYGLTLKTA

SEQ ID NO: 18 - DNA, 1200 bp, Artificial Sequence
  Codon optimized synthetic gene
  CDS (1)..(1200)
  sig_peptide (1)..(81)
  mat_peptide (589)..(1200)
atgaagaaaccgttggggaaaattgtcgcaagcaccgcactactcatttctgttgcttttagttcatcgatcgcatcggctgctacatctgcagctggtggcccagaaccatcaactggcccacttgctacagattctggcgcttcagttgccgagatgtcagcacgctggcttgcgaaagaacacgatctttcaattgagactgcacgtgagcgcatcgctagccaggaagacaaatctcgcaaggctgaagctcttgaacgctcacttggcgctcgtgctgttggcagctttatcgaccaaactggcggtgtattggtagtaaacgttactgatgcggatgcagcagctcgcgttcaaaaggcaggagctacagctcgtgttgttactgaggataaggctgaacttggcgcttctcaagctcgtgctgttaaggctcttggtgccactgtaattgatagctcagttgaccctgtaacgaacaaagttgtagttacagtacctactgctgatgttgcggcagcacgtgcacgtacaagcgacccatctgtaactattcaaggaacagacgcaacggtttctacacaggctaacgtttatggtggccagcagatcgagttctctggatacgtatgttcattaggtttcaacgcaactaaatctggaactcctgttttcatcacagctggccattgtgcggaaggtaaccagactttcactcgtaatggtacaacattgggtacaacacgcggttggtcttttccaggtaacgattatgcgtactcatctcttacttcttcttggactggtattggagctgttgacttatggaatggaacatcagctcgctctgtaactggctcatcaaacgctgctgttggaactgcaatttgcaaatctggtcgtacaacgggatggacatgtggttctgtacaaacgaaaaacgtaactgtaaactataacaacggagatggtacatattctactgtatctggtcttacaaaaagcaatacttgcactgaaggtggagattcaggcggttcttggatggctggcaacttagcacaaggtgtaactagcggtggtgctggctatggtagcaatggagtatgtggccagaaagtaggtcaaccgaacattgcttactttcagcctatcggtgaaatcttgtctgtttatggtcttacattgaaaacagct

SEQ ID NO: 19 - protein, 400 aa, Artificial Sequence
  Synthetic Construct
MKKPLGKIVASTALLISVAFSSSIASAATSAAGGPEPSTGPLATDSGASVAEMSARWLAKEHDLSIETARERIASQEDKSRKAEALERSLGARAVGSFIDQTGGVLVVNVTDADAAARVQKAGATARVVTEDKAELGASQARAVKALGATVIDSSVDPVTNKVVVTVPTADVAAARARTSDPSVTIQGTDATVSTQANVYGGQQIEFSGYVCSLGFNATKSGTPVFITAGHCAEGNQTFTRNGTTLGTTRGWSFPGNDYAYSSLTSSWTGIGAVDLWNGTSARSVTGSSNAAVGTAICKSGRTTGWTCGSVQTKNVTVNYNNGDGTYSTVSGLTKSNTCTEGGDSGGSWMAGNLAQGVTSGGAGYGSNGVCGQKVGQPNIAYFQPIGEILSVYGLTLKTA

SEQ ID NO: 20 - protein, 204 aa, Knoellia flava
  mat_peptide (1)..(204)
ANVYGGQQIEFSGYVCSLGFNATKSGTPVFITAGHCAEGNQTFTRNGTTLGTTRGWSFPGNDYAYSSLTSSWTGIGAVDLWNGTSARSVTGSSNAAVGTAICKSGRTTGWTCGSVQTKNVTVNYNNGDGTYSTVSGLTKSNTCTEGGDSGGSWMAGNLAQGVTSGGAGYGSNGVCGQKVGQPNIAYFQPIGEILSVYGLTLKTA